European Patent Application EP 4 545 555 A1, published April 30, 2025. Title: Recombinant proteins and their use in cancer therapy. Applicant: Real Deal Milk S.L. Application EP. The sequence listing filed with the application follows.

SEQUENCE LISTING (21 sequences)

SEQ ID NO: 1 - protein, 14 aa, Bos taurus
HPHPHLSFMAIPPK

SEQ ID NO: 2 - protein, 27 aa, synthetic construct
  SITE 1: note = X is A or I or L or V
  SITE 4: note = X is D or E
  SITE 6..8: note = X is S or T
  SITE 11: note = X is A or I or L or V
  SITE 12: note = X is D or E
  SITE 13..14: note = X is A or I or L or V
  SITE 15: note = X is D or E
  SITE 17: note = X is S or T
  SITE 18..19: note = X is A or I or L or V
  SITE 20: note = X is S or T
  SITE 21: note = X is A or I or L or V
  SITE 22: note = X is D or E
  SITE 23: note = X iS A or I or L or V
  SITE 24: note = X is S or T
  SITE 26: note = X is D or E
  SITE 27: note = X is A or I or L or V
XSGXPXXXPTXXXXXSXXXXXXXXPXX

SEQ ID NO: 3 - protein, 44 aa, synthetic construct
  SITE 1: note = X is A, L, I or V
  SITE 4: note = X is D or E
  SITE 6..8: note = X is S or T
  SITE 11: note = X is A, I, L or V
  SITE 12: note = X is D or E
  SITE 13..14: note = X is A, I, L or V
  SITE 15: note = X is D or E
  SITE 17: note = X is S or T
  SITE 18..19: note = X is A, I, L or V
  SITE 20: note = X is S or T
  SITE 22: note = X is D or E
  SITE 24: note = X is S or T
  SITE 27..28: note = X is A, I, L, or V
  SITE 21: note = Xis A, I, L or V
  SITE 23: note = X is A, I, L or V
  SITE 26: note = X is D or E
  SITE 29: note = X is D or E
  SITE 33: note = X is D or E
  SITE 34: note = X is A, I, L or V
  SITE 37: note = X is A, I, L or V
  SITE 39: note = X is A, I, L or V
  SITE 40: note = X is S or T
  SITE 43..44: note = X is A, I, L or V
XSGXPXXXPTXXXXXSXXXXXXXXPXXXXSPPXXNTXQXXSTXX

SEQ ID NO: 4 - protein, 41 aa, synthetic construct
  SITE 4: note = X is D or E
  SITE 7: note = X is D or E
  SITE 8: note = X is A, I, L or V
  SITE 10: note = X is S or T
  SITE 11: note = X is A, I, L or V
  SITE 14..15: note = X is A, I, L or V
  SITE 18: note = X is D or E
  SITE 20..22: note = X is S or T
  SITE 25: note = X is A, I, L or V
  SITE 26: note = X is D or E
  SITE 27..28: note = X is A, I, L or V
  SITE 29: note = X is D or E
  SITE 31: note = X is S or T
  SITE 32..33: note = X is A, I, L or V
  SITE 34: note = X is S or T
  SITE 35: note = X is A, I, L or V
  SITE 36: note = X is D or E
  SITE 37: note = X is A, I, L or V
  SITE 38: note = X is S or T
  SITE 40: note = X is D or E
  SITE 41: note = X is A, I, L or V
KNQXKTXXPXXNTXXSGXPXXXPTXXXXXSXXXXXXXXPXX

SEQ ID NO: 5 - protein, 58 aa, synthetic construct
  SITE 4: note = X is D or E
  SITE 7: note = X is D or E
  SITE 8: note = X is A, I, L or V
  SITE 10: note = X is S or T
  SITE 11: note = X is A, I, L, or V
  SITE 14..15: note = X is A, I, L, or V
  SITE 18: note = X is D or E
  SITE 20..22: note = X is S or T
  SITE 25: note = X is A, I, L or V
  SITE 26: note = X is D or E
  SITE 27..28: note = X is A, I, L or V
  SITE 29: note = X is D or E
  SITE 31: note = X is S or T
  SITE 32..33: note = X is A, I, L or V
  SITE 34: note = X is S or T
  SITE 35: note = X is A, I, L or V
  SITE 36: note = X is D or E
  SITE 37: note = X is A, I, L or V
  SITE 38: note = X is S or T
  SITE 40: note = X is D or E
  SITE 41: note = X is A, I, L or V
  SITE 42: note = X is A, I, L or V
  SITE 43: note = X is D or E
  SITE 47: note = X is D or E
  SITE 48: note = X is A, I, L, or V
  SITE 51: note = X is A, I, L or V
  SITE 53: note = X is A, I, L or V
  SITE 54: note = X is S or T
  SITE 57..58: note = X is A, I, L or V
KNQXKTXXPXXNTXXSGXPXXXPTXXXXXSXXXXXXXXPXXXXSPPXXNTXQXXSTXX

SEQ ID NO: 6 - protein, 27 aa, synthetic construct
ASGEPTSTPTIEAVESTVATLEASPEV

SEQ ID NO: 7 - protein, 44 aa, synthetic construct
ASGEPTSTPTIEAVESTVATLEASPEVIESPPEINTVQVTSTAV

SEQ ID NO: 8 - protein, 41 aa, synthetic construct
KNQDKTEIPTINTIASGEPTSTPTIEAVESTVATLEASPEV

SEQ ID NO: 9 - protein, 58 aa, synthetic construct
KNQDKTEIPTINTIASGEPTSTPTIEAVESTVATLEASPEVIESPPEINTVQVTSTAV

SEQ ID NO: 10 - protein, 8 aa, synthetic construct
  SITE 5: note = X is L, M or F
HLSFXAIP

SEQ ID NO: 11 - protein, 14 aa, synthetic construct
  SITE 14: note = X is W, Y, F, C, R, I, M, H, L, V, K, N, T or A
FLQKQQYGISSKFX

SEQ ID NO: 12 - protein, 14 aa, synthetic construct
RPRPRPSFIAIPPK

SEQ ID NO: 13 - protein, 248 aa, synthetic construct
EAEALIVTQTMKGLDIQKVAGTWYSLAMAASDISLLDAQSAPLRVYVEELKPTPEGDLEILLQKWENGECAQKKIIAEKTKIPAVFKIDALNENKVLVLDTDYKKYLLFCMENSAEPEQSLACQCLVRTPEVDDEALEKFDKALKALPMHIRLSFNPTQLEEQCHIHPHPHLSFMAIPPKKNQDKTEIPTINTIASGEPTSTPTIEAVESTVATLEASPEVIESPPEINTVQVTSTAVGSGSHHHHHH

SEQ ID NO: 14 - DNA, 960 bp, synthetic construct
  source 1..960: mol_type = other DNA
atgagatttccatctattttcactgctgttttgtttgctgcttcttctgctttggctgctccagttaacactactactgaagatgagactgctcaaattcctgctgaagctgttattggttactctgatttggagggagattttgatgttgctgttttgcctttctctgcttctatcgctgctaaggaagagggtgtttctttggaaaagagagaagctgaggctttgattgttactcaaactatgaagggtttggatatccaaaaggttgctggtacttggtactctttggctatggctgcttctgatatttctttgttggatgctcaatctgctccattgagagtttatgttgaagagttgaaaccaactcctgaaggagatttggaaattttgttgcaaaagtgggaaaacggagagtgtgctcaaaagaaaattatcgctgaaaagactaagatccctgctgtttttaaaatcgatgctttgaacgagaataaggttttggttttggatactgattacaagaaatatttgttgttctgtatggaaaactctgctgaaccagagcaatctttggcttgtcaatgtttggttagaactcctgaagttgatgatgaagctttggagaagtttgataaagctttgaaggctttgccaatgcatatcagattgtctttcaatcctactcaattggaagagcaatgtcacattcatccacaccctcatttgtctttcatggctattccacctaagaaaaaccaagataagactgaaatcccaactattaatactattgcttctggagagccaacttctactcctactattgaagctgttgagtctactgttgctactttggaagcttctcctgaagttattgagtctccacctgagattaatactgttcaagttacttctactgctgttggttctggatcccatcaccatcaccatcactaa

SEQ ID NO: 15 - protein, 247 aa, synthetic construct
EAEALIVTQTMKGLDIQKVAGTWYNLAMAANDINLLDAQNAPLRVYVEELKPTPEGDLEILLQKWENGECAQKKIIAEKTKIPAVFKIDALNENKVLVLDTDYKKYLLFCMENNAEPEQNLACQCLVRTPEVDDEALEKFDKALKALPMHIRLNFNPTQLEEQCHIHPHPHLTFMAIPPKKNQDKTEIPTINTIATGEPTTTPTIEAVETTVATLEATPEVIETPPEINTVQVTTTAVGGGHHHHHH

SEQ ID NO: 16 - DNA, 957 bp, synthetic construct
  source 1..957: mol_type = other DNA
atgagatttccatctattttcactgctgttttgtttgctgcttcttctgctttggctgctccagttaacactactactgaagatgagactgctcaaattcctgctgaagctgttattggttactctgatttggagggagattttgatgttgctgttttgcctttctctgcttctatcgctgctaaggaagagggtgtttctttggaaaagagagaagctgaggctttgattgttactcaaactatgaagggtttggatatccaaaaggttgctggtacttggtacaacttggctatggctgctaacgatattaacttgttggatgctcaaaacgctccattgagagtttatgttgaagagttgaaaccaactcctgaaggagatttggaaattttgttgcaaaagtgggaaaacggagagtgtgctcaaaagaaaattatcgctgaaaagactaagatccctgctgtttttaaaatcgatgctttgaacgagaataaggttttggttttggatactgattacaagaaatatttgttgttctgtatggaaaacaacgctgaaccagagcaaaacttggcttgtcaatgtttggttagaactcctgaagttgatgatgaagctttggagaagtttgataaagctttgaaggctttgccaatgcatatcagattgaacttcaatcctactcaattggaagagcaatgtcacattcatccacaccctcatttgactttcatggctattccacctaagaaaaaccaagataagactgaaatcccaactattaatactattgctactggagagccaactactactcctactattgaagctgttgagactactgttgctactttggaagctactcctgaagttattgagactccacctgagattaatactgttcaagttactactactgctgttggtggaggtcatcaccatcaccatcactaa

SEQ ID NO: 17 - protein, 248 aa, synthetic construct
EAEALIVTQTMKGLDIQKVAGTWYSLAMAASDISLLDAQSAPLRVYVEELKPTPEGDLEILLQKWENGEVAQKKIIAEKTKIPAVFKIDALNENKVLVLDTDYKKYLLFAMENSAEPEQSLAVQALVRTPEVDDEALEKFDKALKALPMHIRLSFNPTQLEEQAHIHPHPHLSFMAIPPKKNQDKTEIPTINTIASGEPTSTPTIEAVESTVATLEASPEVIESPPEINTVQVTSTAVGSGSHHHHHH

SEQ ID NO: 18 - DNA, 960 bp, synthetic construct
  source 1..960: mol_type = other DNA
atgagatttccatctattttcactgctgttttgtttgctgcttcttctgctttggctgctccagttaacactactactgaagatgagactgctcaaattcctgctgaagctgttattggttactctgatttggagggagattttgatgttgctgttttgcctttctctgcttctatcgctgctaaggaagagggtgtttctttggaaaagagagaagctgaggctttgattgttactcaaactatgaagggtttggatatccaaaaggttgctggtacttggtactctttggctatggctgcttctgatatttctttgttggatgctcaatctgctccattgagagtttatgttgaagagttgaaaccaactcctgaaggagatttggaaattttgttgcaaaagtgggaaaacggagaggttgctcaaaagaaaattatcgctgaaaagactaagatccctgctgtttttaaaatcgatgctttgaacgagaataaggttttggttttggatactgattacaagaaatatttgttgttcgctatggaaaactctgctgaaccagagcaatctttggctgttcaagctttggttagaactcctgaagttgatgatgaagctttggagaagtttgataaagctttgaaggctttgccaatgcatatcagattgtctttcaatcctactcaattggaagagcaagctcacattcatccacaccctcatttgtctttcatggctattccacctaagaaaaaccaagataagactgaaatcccaactattaatactattgcttctggagagccaacttctactcctactattgaagctgttgagtctactgttgctactttggaagcttctcctgaagttattgagtctccacctgagattaatactgttcaagttacttctactgctgttggttctggatcccatcaccatcaccatcactaa

SEQ ID NO: 19 - protein, 248 aa, synthetic construct
EAEALIVTQTLKGLDIQKVAGTWYSLALAASDISLLDAQSAPLRVYVEELKPTPEGDLEILLQKWENGECAQKKIIAEKTKIPAVFKIDALNENKVLVLDTDYKKYLLFCLENSAEPEQSLACQCLVRTPEVDDEALEKFDKALKALPLHIRLSFNPTQLEEQCHIHPHPHLSFMAIPPKKNQDKTEIPTINTIASGEPTSTPTIEAVESTVATLEASPEVIESPPEINTVQVTSTAVGSGSHHHHHH

SEQ ID NO: 20 - DNA, 960 bp, synthetic construct
  source 1..960: mol_type = other DNA
atgagatttccatctattttcactgctgttttgtttgctgcttcttctgctttggctgctccagttaacactactactgaagatgagactgctcaaattcctgctgaagctgttattggttactctgatttggagggagattttgatgttgctgttttgcctttctctgcttctatcgctgctaaggaagagggtgtttctttggaaaagagagaagctgaggctttgattgttactcaaactttgaagggtttggatatccaaaaggttgctggtacttggtactctttggctttggctgcttctgatatttctttgttggatgctcaatctgctccattgagagtttatgttgaagagttgaaaccaactcctgaaggagatttggaaattttgttgcaaaagtgggaaaacggagagtgtgctcaaaagaaaattatcgctgaaaagactaagatccctgctgtttttaaaatcgatgctttgaacgagaataaggttttggttttggatactgattacaagaaatatttgttgttctgtttggaaaactctgctgaaccagagcaatctttggcttgtcaatgtttggttagaactcctgaagttgatgatgaagctttggagaagtttgataaagctttgaaggctttgccattgcatatcagattgtctttcaatcctactcaattggaagagcaatgtcacattcatccacaccctcatttgtctttcatggctattccacctaagaaaaaccaagataagactgaaatcccaactattaatactattgcttctggagagccaacttctactcctactattgaagctgttgagtctactgttgctactttggaagcttctcctgaagttattgagtctccacctgagattaatactgttcaagttacttctactgctgttggttctggatcccatcaccatcaccatcactaa

SEQ ID NO: 21 - protein, 10 aa, synthetic construct
GSGSHHHHHH